European Patent Application EP 4 711 460 A1, published March 18, 2026. Title: DNA aptamer that selectively binds to soluble FLT-1 and carrier supporting thereof. Applicant: TAGCYX Biotechnologies Inc. The sequence listing filed with the application follows.

SEQUENCE LISTING (9 sequences)

SEQ ID NO: 1 - DNA, 92 bp, synthetic construct
  source 1..92: mol_type = other DNA
  misc_feature 34: note = n is synthetic base; Ds (7-(2-thienyl)imidazo[4,5-b]pyridine)
  misc_feature 53: note = n is synthetic base; Ds (7-(2-thienyl)imidazo[4,5-b]pyridine)
atcacgtcagcgaaattaaatcgagggacccggntgaaagcgccgccaacggntgaggggtctttccgatacaatcctgatccatgagacgg

SEQ ID NO: 2 - DNA, 92 bp, synthetic construct
  source 1..92: mol_type = other DNA
  misc_feature 48: note = n is synthetic base; Ds (7-(2-thienyl)imidazo[4,5-b]pyridine)
  misc_feature 34: note = n is synthetic base; Ds (7-(2-thienyl)imidazo[4,5-b]pyridine)
atcacgtcagcgaaattaaatcgagcgacccccngcgccgccgaaggntgaggggacgggggagctagatacaatcctgatccatgagacgg

SEQ ID NO: 3 - DNA, 92 bp, synthetic construct
  source 1..92: mol_type = other DNA
  misc_feature 46: note = n is synthetic base; Ds (7-(2-thienyl)imidazo[4,5-b]pyridine)
  misc_feature 37: note = n is synthetic base; Ds(7-(2-thienyl)imidazo[4,5-b]pyridine)
ttgtgcagtcgctctaatttagctctacccgcttaangattgttangttgtacgaaacgcattcggggttggaatcttaagtgaagtcgcgc

SEQ ID NO: 4 - DNA, 44 bp, synthetic construct
  source 1..44: mol_type = other DNA
  misc_feature 31: note = n is synthetic base; Ds (7-(2-thienyl)imidazo[4,5-b]pyridine)
  misc_feature 12: note = n is synthetic base; Ds(7-(2-thienyl)imidazo[4,5-b]pyridine)
gagggacccggntgaaagcgccgccaacggntgaggggtctttc

SEQ ID NO: 5 - DNA, 34 bp, synthetic construct
  source 1..34: mol_type = other DNA
  misc_feature 6: note = n is synthetic base; Ds (7-(2-thienyl)imidazo[4,5-b]pyridine)
  misc_feature 20: note = n is synthetic base; Ds (7-(2-thienyl)imidazo[4,5-b]pyridine)
cccccngcgccgccgaaggntgaggggacggggg

SEQ ID NO: 6 - DNA, 43 bp, synthetic construct
  source 1..43: mol_type = other DNA
  misc_feature 20: note = n is synthetic base; Ds (7-(2-thienyl)imidazo[4,5-b]pyridine)
  misc_feature 39: note = n is an artificial base
  misc_feature 6: note = n is synthetic base; Ds(7-(2-thienyl)imidazo[4,5-b]pyridine)
cgcccngcgccgccgaaggntgaggggacgggcgcgcgnagcg

SEQ ID NO: 7 - DNA, 47 bp, synthetic construct
  source 1..47: mol_type = other DNA
  misc_feature 22: note = n is synthetic base; Ds (7-(2-thienyl)imidazo[4,5-b]pyridine)
  misc_feature 43: note = n is an artificial base
  misc_feature 8: note = n is synthetic base; Ds(7-(2-thienyl)imidazo[4,5-b]pyridine)
ctgacccngcgccgccgaaggntgaggggacgggtcagcgcgnagcg

SEQ ID NO: 8 - DNA, 47 bp, synthetic construct
  source 1..47: mol_type = other DNA
  misc_feature 22: note = n is synthetic base; Ds (7-(2-thienyl)imidazo[4,5-b]pyridine)
  misc_feature 8: note = n is synthetic base; Ds(7-(2-thienyl)imidazo[4,5-b]pyridine)
ctgacccngcgccgccgaaggntgaggggacgggtcagcgcgaagcg

SEQ ID NO: 9 - DNA, 30 bp, synthetic construct
  source 1..30: mol_type = other DNA
  misc_feature 18: note = n is synthetic base; Ds (7-(2-thienyl)imidazo[4,5-b]pyridine)
  misc_feature 4: note = n is synthetic base; Ds(7-(2-thienyl)imidazo[4,5-b]pyridine)
ccgngcgccgccgaaggntgaggggaccgg